European Patent Application EP 4 464 718 A1, published November 20, 2024. Title: Variants of L-threonine efflux protein and L-threonine production method using the same. Applicant: CJ CheilJedang Corporation. The sequence listing filed with the application follows.

SEQUENCE LISTING (23 sequences)

SEQ ID NO: 1 - protein, 206 aa, Escherichia coli
  REGION 1..206: note = rhtC(WT) AA
MLMLFLTVAMVHIVALMSPGPDFFFVSQTAVSRSRKEAMMGVLGITCGVMVWAGIALLGLHLIIEKMAWLHTLIMVGGGLYLCWMGYQMLRGALKKEAVSAPAPQVELAKSGRSFLKGLLTNLANPKAIIYFGSVFSLFVGDNVGTTARWGIFALIIVETLAWFTVVASLFALPQMRRGYQRLAKWIDGFAGALFAGFGIHLIISR

SEQ ID NO: 2 - DNA, 621 bp, Escherichia coli
  misc_feature 1..621: note = rhtC(WT) NT
  source 1..621: mol_type = genomic DNA
atgttgatgttatttctcaccgtcgccatggtgcacattgtggcgcttatgagccccggtcccgatttcttttttgtctctcagaccgctgtcagtcgttcccgtaaagaagcgatgatgggcgtgctgggcattacctgcggcgtaatggtttgggctgggattgcgctgcttggcctgcatttgattatcgaaaaaatggcctggctgcatacgctgattatggtgggcggtggcctgtatctctgctggatgggttaccagatgctacgtggtgcactgaaaaaagaggcggtttctgcacctgcgccacaggtcgagctggcgaaaagtgggcgcagtttcctgaaaggtttactgaccaatctcgctaatccgaaagcgattatctactttggctcggtgttctcattgtttgtcggtgataacgttggcactaccgcgcgctggggcatttttgcgctgatcattgtcgaaacgctggcgtggtttaccgtcgttgccagcctgtttgccctgccgcaaatgcgccgtggttatcaacgtctggcgaagtggattgatggttttgccggggcgttatttgccggatttggcattcatttgattatttcgcggtga

SEQ ID NO: 3 - protein, 206 aa, synthetic construct
  REGION 1..206: note = rhtC(G133S) AA
MLMLFLTVAMVHIVALMSPGPDFFFVSQTAVSRSRKEAMMGVLGITCGVMVWAGIALLGLHLIIEKMAWLHTLIMVGGGLYLCWMGYQMLRGALKKEAVSAPAPQVELAKSGRSFLKGLLTNLANPKAIIYFSSVFSLFVGDNVGTTARWGIFALIIVETLAWFTVVASLFALPQMRRGYQRLAKWIDGFAGALFAGFGIHLIISR

SEQ ID NO: 4 - DNA, 621 bp, synthetic construct
  misc_feature 1..621: note = rhtC(G133S) NT_AGC
  source 1..621: mol_type = other DNA
atgttgatgttatttctcaccgtcgccatggtgcacattgtggcgcttatgagccccggtcccgatttcttttttgtctctcagaccgctgtcagtcgttcccgtaaagaagcgatgatgggcgtgctgggcattacctgcggcgtaatggtttgggctgggattgcgctgcttggcctgcatttgattatcgaaaaaatggcctggctgcatacgctgattatggtgggcggtggcctgtatctctgctggatgggttaccagatgctacgtggtgcactgaaaaaagaggcggtttctgcacctgcgccacaggtcgagctggcgaaaagtgggcgcagtttcctgaaaggtttactgaccaatctcgctaatccgaaagcgattatctactttagctcggtgttctcattgtttgtcggtgataacgttggcactaccgcgcgctggggcatttttgcgctgatcattgtcgaaacgctggcgtggtttaccgtcgttgccagcctgtttgccctgccgcaaatgcgccgtggttatcaacgtctggcgaagtggattgatggttttgccggggcgttatttgccggatttggcattcatttgattatttcgcggtga

SEQ ID NO: 5 - DNA, 621 bp, synthetic construct
  misc_feature 1..621: note = rhtC(G133S) NT_AGT
  source 1..621: mol_type = other DNA
atgttgatgttatttctcaccgtcgccatggtgcacattgtggcgcttatgagccccggtcccgatttcttttttgtctctcagaccgctgtcagtcgttcccgtaaagaagcgatgatgggcgtgctgggcattacctgcggcgtaatggtttgggctgggattgcgctgcttggcctgcatttgattatcgaaaaaatggcctggctgcatacgctgattatggtgggcggtggcctgtatctctgctggatgggttaccagatgctacgtggtgcactgaaaaaagaggcggtttctgcacctgcgccacaggtcgagctggcgaaaagtgggcgcagtttcctgaaaggtttactgaccaatctcgctaatccgaaagcgattatctactttagttcggtgttctcattgtttgtcggtgataacgttggcactaccgcgcgctggggcatttttgcgctgatcattgtcgaaacgctggcgtggtttaccgtcgttgccagcctgtttgccctgccgcaaatgcgccgtggttatcaacgtctggcgaagtggattgatggttttgccggggcgttatttgccggatttggcattcatttgattatttcgcggtga

SEQ ID NO: 6 - DNA, 500 bp, synthetic construct
  misc_feature 1..500: note = PrhtC
  source 1..500: mol_type = other DNA
gccatgaacattgggtgagcgtgatccgccagctgattcacctcggcctggtgacgcaaaatattgcccagcattctgccctacaactgacagaggccgcgcgcccggtgctgcgcggcgaatcctctttgcaacttgccgtgccgcgtatcgtggcgctcaaaccgaaagcgatgcagaaatcgttcggcggcaactatgatcgcaaactgttcgccaaattacgcaaactgcgtaaatcgatagccgatgaaagtaatgtcccgccgtacgtggtgtttaacgacgcaaccttgattgagatggctgaacagatgccgatcaccgccagcgaaatgctcagcgttaacggcgttgggatgcgcaagctggaacgctttggcaaaccgtttatggcgctgattcgtgcgcatgttgatggcgatgacgaagagtagtcagcagcataaaaaagtgccagtatgaagactccgtaaacgtttcccccgcgagtcaaatgt

SEQ ID NO: 7 - DNA, 40 bp, synthetic construct
  misc_feature 1..40: note = PrhtC F
  source 1..40: mol_type = other DNA
tcgagctcggtacccggggagccatgaacattgggtgagc

SEQ ID NO: 8 - DNA, 40 bp, synthetic construct
  misc_feature 1..40: note = PrhtC R
  source 1..40: mol_type = other DNA
gtcgactctagaggaggatccacatttgactcgcggggga

SEQ ID NO: 9 - DNA, 44 bp, synthetic construct
  misc_feature 1..44: note = rhtC F
  source 1..44: mol_type = other DNA
tcccccgcgagtcaaatgtgatgttgatgttatttctcaccgtc

SEQ ID NO: 10 - DNA, 45 bp, synthetic construct
  misc_feature 1..45: note = rhtC R
  source 1..45: mol_type = other DNA
gtcgactctagaggaggatctcaccgcgaaataatcaaatgaatg

SEQ ID NO: 11 - DNA, 40 bp, synthetic construct
  misc_feature 1..40: note = 1762A F
  source 1..40: mol_type = other DNA
tgaattcgagctcggtacccgtggccagtattaatgggct

SEQ ID NO: 12 - DNA, 40 bp, synthetic construct
  misc_feature 1..40: note = 1762A R
  source 1..40: mol_type = other DNA
gtctcaagcagagactcgagcaccctcaatgggtcaggcc

SEQ ID NO: 13 - DNA, 40 bp, synthetic construct
  misc_feature 1..40: note = 1762B F
  source 1..40: mol_type = other DNA
acccattgagggtgctcgagtctctgcttgagacttaagc

SEQ ID NO: 14 - DNA, 40 bp, synthetic construct
  misc_feature 1..40: note = 1762B R
  source 1..40: mol_type = other DNA
gtcgactctagaggatccccaggctctctatgggcacctc

SEQ ID NO: 15 - DNA, 40 bp, synthetic construct
  misc_feature 1..40: note = rhtC(m) F
  source 1..40: mol_type = other DNA
gcctgacccattgagggtgcgccatgaacattgggtgagc

SEQ ID NO: 16 - DNA, 50 bp, synthetic construct
  misc_feature 1..50: note = rhtC(m) R
  source 1..50: mol_type = other DNA
ataacgcttaagtctcaagcagagactcgatcaccgcgaaataatcaaat

SEQ ID NO: 17 - DNA, 22 bp, synthetic construct
  misc_feature 1..22: note = pDC F
  source 1..22: mol_type = other DNA
ctattacgccagctggcgaaag

SEQ ID NO: 18 - DNA, 20 bp, synthetic construct
  misc_feature 1..20: note = pDC R
  source 1..20: mol_type = other DNA
atgttgtgtggaattgtgag

SEQ ID NO: 19 - DNA, 20 bp, synthetic construct
  misc_feature 1..20: note = seq 1
  source 1..20: mol_type = other DNA
ttctcttgttcctttctgag

SEQ ID NO: 20 - DNA, 20 bp, synthetic construct
  misc_feature 1..20: note = seq 2
  source 1..20: mol_type = other DNA
ttctgagtagctgagcttcg

SEQ ID NO: 21 - DNA, 20 bp, synthetic construct
  misc_feature 1..20: note = seq 3
  source 1..20: mol_type = other DNA
ccagatgctacgtggtgcac

SEQ ID NO: 22 - DNA, 20 bp, synthetic construct
  misc_feature 1..20: note = seq 4
  source 1..20: mol_type = other DNA
tggtctgctcgcttctcgat

SEQ ID NO: 23 - DNA, 20 bp, synthetic construct
  misc_feature 1..20: note = seq 5
  source 1..20: mol_type = other DNA
tatcttcgtagagcactgct